European Patent Application EP 4 458 967 A1, published November 6, 2024. Title: PHARMACEUTICAL COMPOSITION COMPRISING MULTIPLE SUPPRESSOR TRANSFER RNAS. Applicant: UNIVERSITÄT HAMBURG. The sequence listing filed with the application follows.

SEQUENCE LISTING (78 sequences)

SEQ ID NO: 1 - RNA, 17 nt, synthetic construct
  source 1..17: mol_type = other RNA
  misc_feature 8..10: note = anticodon
gcaggnnnnnnncctgt

SEQ ID NO: 2 - RNA, 17 nt, synthetic construct
  source 1..17: mol_type = other RNA
  misc_feature 8..10: note = anticodon
ttgggnnnnnnnctcaa

SEQ ID NO: 3 - RNA, 17 nt, synthetic construct
  source 1..17: mol_type = other RNA
  misc_feature 8..10: note = anticodon
ttggannnnnnnttcaa

SEQ ID NO: 4 - RNA, 17 nt, synthetic construct
  source 1..17: mol_type = other RNA
  misc_feature 8..10: note = anticodon
atggtnnnnnnnaccat

SEQ ID NO: 5 - RNA, 17 nt, synthetic construct
  source 1..17: mol_type = other RNA
  misc_feature 8..10: note = anticodon
gcggannnnnnntccgc

SEQ ID NO: 6 - RNA, 17 nt, synthetic construct
  source 1..17: mol_type = other RNA
  misc_feature 8..10: note = anticodon
gcggtnnnnnnnaccgc

SEQ ID NO: 7 - RNA, 17 nt, synthetic construct
  source 1..17: mol_type = other RNA
  misc_feature 8..10: note = anticodon
ggcggnnnnnnnccgcc

SEQ ID NO: 8 - RNA, 17 nt, synthetic construct
  source 1..17: mol_type = other RNA
  misc_feature 8..10: note = anticodon
ggcgcnnnnnnngcgcc

SEQ ID NO: 9 - RNA, 17 nt, synthetic construct
  source 1..17: mol_type = other RNA
  misc_feature 8..10: note = anticodon
gcaggctnnnaacctgt

SEQ ID NO: 10 - RNA, 17 nt, synthetic construct
  source 1..17: mol_type = other RNA
  misc_feature 8..10: note = anticodon
ttgggctnnnaactcaa

SEQ ID NO: 11 - RNA, 17 nt, synthetic construct
  source 1..17: mol_type = other RNA
  misc_feature 8..10: note = anticodon
ttggactnnnaattcaa

SEQ ID NO: 12 - RNA, 17 nt, synthetic construct
  source 1..17: mol_type = other RNA
  misc_feature 8..10: note = anticodon
atggtctnnnaaaccat

SEQ ID NO: 13 - RNA, 17 nt, synthetic construct
  source 1..17: mol_type = other RNA
  misc_feature 8..10: note = anticodon
gcggactnnnaatccgc

SEQ ID NO: 14 - RNA, 17 nt, synthetic construct
  source 1..17: mol_type = other RNA
  misc_feature 8..10: note = anticodon
gcggtctnnnaaaccgc

SEQ ID NO: 15 - RNA, 17 nt, synthetic construct
  source 1..17: mol_type = other RNA
  misc_feature 8..10: note = anticodon
ggcggctnnnaaccgcc

SEQ ID NO: 16 - RNA, 17 nt, synthetic construct
  source 1..17: mol_type = other RNA
  misc_feature 8..10: note = anticodon
ggcgcctnnnaagcgcc

SEQ ID NO: 17 - RNA, 12 nt, synthetic construct
  source 1..12: mol_type = other RNA
tggggtttcccc

SEQ ID NO: 18 - RNA, 12 nt, synthetic construct
  source 1..12: mol_type = other RNA
aggggaaacccc

SEQ ID NO: 19 - RNA, 17 nt, synthetic construct
  source 1..17: mol_type = other RNA
  misc_feature 6..12: note = T Loop
gcgggttcgaatcccgt

SEQ ID NO: 20 - RNA, 17 nt, synthetic construct
  source 1..17: mol_type = other RNA
  misc_feature 6..12: note = T loop
acgggttcgaatcccgt

SEQ ID NO: 21 - RNA, 17 nt, synthetic construct
  source 1..17: mol_type = other RNA
  misc_feature 6..12: note = T loop
gcgggttcgagtcccgt

SEQ ID NO: 22 - RNA, 17 nt, synthetic construct
  source 1..17: mol_type = other RNA
  misc_feature 6..12: note = T loop
acgggttcgagtcccgt

SEQ ID NO: 23 - RNA, 17 nt, synthetic construct
  source 1..17: mol_type = other RNA
  misc_feature 6..12: note = T loop
gtaggttcgagtcccat

SEQ ID NO: 24 - RNA, 17 nt, synthetic construct
  source 1..17: mol_type = other RNA
  misc_feature 6..12: note = T loop
gtcggttcgagtccgat

SEQ ID NO: 25 - RNA, 17 nt, synthetic construct
  source 1..17: mol_type = other RNA
  misc_feature 6..12: note = T loop
gccggttcgagtccggt

SEQ ID NO: 26 - RNA, 17 nt, synthetic construct
  source 1..17: mol_type = other RNA
  misc_feature 6..12: note = T loop
gcaggttcgagtcccgt

SEQ ID NO: 27 - RNA, 17 nt, synthetic construct
  source 1..17: mol_type = other RNA
  misc_feature 6..12: note = T loop
gccggttcgagtccggt

SEQ ID NO: 28 - DNA, 17 bp, synthetic construct
  source 1..17: mol_type = other DNA
tgacctaagtgtaaagt

SEQ ID NO: 29 - DNA, 18 bp, synthetic construct
  source 1..18: mol_type = other DNA
tgagatttccttcaggtt

SEQ ID NO: 30 - DNA, 31 bp, synthetic construct
  source 1..31: mol_type = other DNA
tatatagttctgtatgagaccactctttccc

SEQ ID NO: 31 - DNA, 17 bp, synthetic construct
  source 1..17: mol_type = other DNA
accataaacgtgaaatg

SEQ ID NO: 32 - DNA, 18 bp, synthetic construct
  source 1..18: mol_type = other DNA
tctttggatttgggaatc

SEQ ID NO: 33 - DNA, 31 bp, synthetic construct
  source 1..31: mol_type = other DNA
ttataagttctgtatgagaccactctttccc

SEQ ID NO: 34 - DNA, 50 bp, synthetic construct
  source 1..50: mol_type = other DNA
vnanantvhanannttnnnatranattcngdgvgnaanatabtnctvgnd

SEQ ID NO: 35 - DNA, 50 bp, synthetic construct
  source 1..50: mol_type = other DNA
gcnggdggcgngttcbbctgtnvnagcntncgdngncgtttnncntcggt

SEQ ID NO: 36 - DNA, 10 bp, synthetic construct
  source 1..10: mol_type = other DNA
gaaatgcctt

SEQ ID NO: 37 - DNA, 10 bp, synthetic construct
  source 1..10: mol_type = other DNA
gtgggaacta

SEQ ID NO: 38 - DNA, 10 bp, synthetic construct
  source 1..10: mol_type = other DNA
gtgttgcttg

SEQ ID NO: 39 - DNA, 66 bp, synthetic construct
  source 1..66: mol_type = other DNA
tgacctaagtgtaaagttgagatttccttcaggtttatatagttctgtatgagaccactctttccc

SEQ ID NO: 40 - DNA, 66 bp, synthetic construct
  source 1..66: mol_type = other DNA
accataaacgtgaaatgtctttggatttgggaatcttataagttctgtatgagaccactctttccc

SEQ ID NO: 41 - DNA, 66 bp, synthetic construct
  source 1..66: mol_type = other DNA
tgacctaagtgtaaagtnnnnnnnnnnnnnnnnnnnnnnnnnnnnnnnnnnnnnnnnnnnnnnnnn

SEQ ID NO: 42 - DNA, 66 bp, synthetic construct
  source 1..66: mol_type = other DNA
nnnnnnnnnnnnnnnnntgagatttccttcaggttnnnnnnnnnnnnnnnnnnnnnnnnnnnnnnn

SEQ ID NO: 43 - DNA, 66 bp, synthetic construct
  source 1..66: mol_type = other DNA
nnnnnnnnnnnnnnnnnnnnnnnnnnnnnnnnnnntatatagttctgtatgagaccactctttccc

SEQ ID NO: 44 - DNA, 66 bp, synthetic construct
  source 1..66: mol_type = other DNA
tgacctaagtgtaaagttgagatttccttcaggttnnnnnnnnnnnnnnnnnnnnnnnnnnnnnnn

SEQ ID NO: 45 - DNA, 66 bp, synthetic construct
  source 1..66: mol_type = other DNA
nnnnnnnnnnnnnnnnntgagatttccttcaggtttatatagttctgtatgagaccactctttccc

SEQ ID NO: 46 - DNA, 66 bp, synthetic construct
  source 1..66: mol_type = other DNA
tgacctaagtgtaaagtnnnnnnnnnnnnnnnnnntatatagttctgtatgagaccactctttccc

SEQ ID NO: 47 - DNA, 66 bp, synthetic construct
  source 1..66: mol_type = other DNA
accataaacgtgaaatgnnnnnnnnnnnnnnnnnnnnnnnnnnnnnnnnnnnnnnnnnnnnnnnnn

SEQ ID NO: 48 - DNA, 66 bp, synthetic construct
  source 1..66: mol_type = other DNA
nnnnnnnnnnnnnnnnntctttggatttgggaatcnnnnnnnnnnnnnnnnnnnnnnnnnnnnnnn

SEQ ID NO: 49 - DNA, 66 bp, synthetic construct
  source 1..66: mol_type = other DNA
nnnnnnnnnnnnnnnnnnnnnnnnnnnnnnnnnnnttataagttctgtatgagaccactctttccc

SEQ ID NO: 50 - DNA, 66 bp, synthetic construct
  source 1..66: mol_type = other DNA
accataaacgtgaaatgtctttggatttgggaatcnnnnnnnnnnnnnnnnnnnnnnnnnnnnnnn

SEQ ID NO: 51 - DNA, 66 bp, synthetic construct
  source 1..66: mol_type = other DNA
nnnnnnnnnnnnnnnnntctttggatttgggaatcttataagttctgtatgagaccactctttccc

SEQ ID NO: 52 - DNA, 66 bp, synthetic construct
  source 1..66: mol_type = other DNA
accataaacgtgaaatgnnnnnnnnnnnnnnnnnnttataagttctgtatgagaccactctttccc

SEQ ID NO: 53 - DNA, 66 bp, synthetic construct
  source 1..66: mol_type = other DNA
tgacctaagtgtaaagttctttggatttgggaatcnnnnnnnnnnnnnnnnnnnnnnnnnnnnnnn

SEQ ID NO: 54 - DNA, 66 bp, synthetic construct
  source 1..66: mol_type = other DNA
tgacctaagtgtaaagtnnnnnnnnnnnnnnnnnnttataagttctgtatgagaccactctttccc

SEQ ID NO: 55 - DNA, 66 bp, synthetic construct
  source 1..66: mol_type = other DNA
nnnnnnnnnnnnnnnnntgagatttccttcaggttttataagttctgtatgagaccactctttccc

SEQ ID NO: 56 - DNA, 66 bp, synthetic construct
  source 1..66: mol_type = other DNA
accataaacgtgaaatgtgagatttccttcaggttnnnnnnnnnnnnnnnnnnnnnnnnnnnnnnn

SEQ ID NO: 57 - DNA, 66 bp, synthetic construct
  source 1..66: mol_type = other DNA
nnnnnnnnnnnnnnnnntctttggatttgggaatctatatagttctgtatgagaccactctttccc

SEQ ID NO: 58 - DNA, 66 bp, synthetic construct
  source 1..66: mol_type = other DNA
accataaacgtgaaatgnnnnnnnnnnnnnnnnnntatatagttctgtatgagaccactctttccc

SEQ ID NO: 59 - DNA, 66 bp, synthetic construct
  source 1..66: mol_type = other DNA
tgacctaagtgtaaagttctttggatttgggaatcttataagttctgtatgagaccactctttccc

SEQ ID NO: 60 - DNA, 66 bp, synthetic construct
  source 1..66: mol_type = other DNA
accataaacgtgaaatgtgagatttccttcaggttttataagttctgtatgagaccactctttccc

SEQ ID NO: 61 - DNA, 66 bp, synthetic construct
  source 1..66: mol_type = other DNA
accataaacgtgaaatgtctttggatttgggaatctatatagttctgtatgagaccactctttccc

SEQ ID NO: 62 - DNA, 66 bp, synthetic construct
  source 1..66: mol_type = other DNA
tgacctaagtgtaaagttgagatttccttcaggttttataagttctgtatgagaccactctttccc

SEQ ID NO: 63 - DNA, 66 bp, synthetic construct
  source 1..66: mol_type = other DNA
tgacctaagtgtaaagttctttggatttgggaatctatatagttctgtatgagaccactctttccc

SEQ ID NO: 64 - DNA, 66 bp, synthetic construct
  source 1..66: mol_type = other DNA
accataaacgtgaaatgtgagatttccttcaggtttatatagttctgtatgagaccactctttccc

SEQ ID NO: 65 - DNA, 50 bp, synthetic construct
  source 1..50: mol_type = other DNA
ccatgatcccccactattaaggatatccggagaggatgctacctatcagg

SEQ ID NO: 66 - DNA, 50 bp, synthetic construct
  source 1..50: mol_type = other DNA
agaccagctgtatagcctcagaatgatccgtccggaaacccttactaggt

SEQ ID NO: 67 - DNA, 50 bp, synthetic construct
  source 1..50: mol_type = other DNA
gcatattgcagaacttgtgaagaggctttatgcgccacacactgcaagca

SEQ ID NO: 68 - DNA, 50 bp, synthetic construct
  source 1..50: mol_type = other DNA
gcaaaagcaaaagcattaagtagctttctggcataaacatattgcagctg

SEQ ID NO: 69 - DNA, 50 bp, synthetic construct
  source 1..50: mol_type = other DNA
ggttgcggtaagcattagagggctatcagcagcatcttatcgcagcggag

SEQ ID NO: 70 - DNA, 50 bp, synthetic construct
  source 1..50: mol_type = other DNA
ctgcagtataaccttgaagtaccatcacggagagaaacagtgccatctca

SEQ ID NO: 71 - DNA, 50 bp, synthetic construct
  source 1..50: mol_type = other DNA
aacgactacgtagtgttctataacaatcatgagaaattttagttctagat

SEQ ID NO: 72 - DNA, 50 bp, synthetic construct
  source 1..50: mol_type = other DNA
gctggtggcgagttccgctgtgccagcttccgttggcgtttgccatcggt

SEQ ID NO: 73 - DNA, 50 bp, synthetic construct; identical to SEQ ID NO: 72
  source 1..50: mol_type = other DNA

SEQ ID NO: 74 - DNA, 50 bp, synthetic construct; identical to SEQ ID NO: 72
  source 1..50: mol_type = other DNA

SEQ ID NO: 75 - DNA, 50 bp, synthetic construct
  source 1..50: mol_type = other DNA
atgcggccttgtgtggtggctcattgtggtgggccagaaaacgcgtgcaa

SEQ ID NO: 76 - DNA, 50 bp, synthetic construct
  source 1..50: mol_type = other DNA
gccagaggcgctggggccaggaggcgcaagccgggccctgaagccgcctc

SEQ ID NO: 77 - DNA, 50 bp, synthetic construct
  source 1..50: mol_type = other DNA
aaagaaattaggaaattcctgtggaagctggcgcgttgatgcacttcgtc

SEQ ID NO: 78 - DNA, 50 bp, synthetic construct
  source 1..50: mol_type = other DNA
caacaaacattttgcttttttaaaattgaaagaacaactgttttccgggt